European Patent Specification EP 3 337 895 B1, published March 25, 2026. Title: Enhanced Recombination of Genomic Loci. Applicant: Monsanto Technology LLC Caldwell, David G Nagy, Ervin. The sequence listing filed with the application follows.

SEQUENCE LISTING (82 sequences)

SEQ ID NO: 1 - DNA, 3885 bp, Zea maize
atggcggacttggcgctagttggcttaaggtgggcagcatcgccgattgtcaaggagcttcttactaaagcttcagcttacctcagtgtggacatggtgcgtgagatcgaacgactacaagacactgtcctgccacagttcgagttggtgattcaagcggcccagaagagcccccataggggcaagctggaatcctggcttcggcgtctcaaagaagccttctatgatgccgaggacctgctggacgagcatgagtacaacgtccttaaggccaaggccaagagcggaaaaggtcccctgctccgagaggatgaaagctcctccactgcaaccactgtcatgaagccttttcattctgctatgaacagggcacgcaacttgctccctgggaacagaaggctaattagcaagatgaacgagctcaaagctatcctgacagaagcccaacaacttcgagatcttcttggcttgccacatggcaataccgtcgagtgcccagctgcagcacctaccagtgttcccacaaccacatcacttcccacttccaaggttttcggtcgcgacagggatcgtgatcgcatagtaaaatttcttctcggcaagacaacaactgctgaggcaagctcaactaagtactccggtttggccattgttggattgggaggaatggggaagtctaccttagcacaatatgtctataatgacaagaggattgaagaatgctttgatgtcaggatgtggatctgtatctcgcgcaaacttgatgtgcatcgtcacacaagggagattatagagtctgcaaaaaagggagagtgcccacgtgttgataatctcgatactctccagtgcaaattacgtgatatactacaagagtcacagaaattcctgcttgtcttggatgatgtttggtttgaaaaatctcatagtgagacagagtgggagttattccttgctccattagtctctaaacagtcagggagcaaagttttggttacttctcaaagtggaacacttccggccgctatttgttgtgaacaagaacatgtcattcatttggaaaacatggatgatactgagtttttggctctttttaaacaccatgctttctctggagcagaaatcaaagaccaactgttacgcacgaagctggaagacactgcagaggagattgctaaaaggcttggacaatgtcctttggcagcaaaagttctgggttctcgattgtgcaggaaaaaggatattgctgaatggaaagctgctctaaagcttggagatttaagtgatcccttcacatctctgttgtggagttacgagaagttagatccacgtctgcagaggtgcttcttgtattgcagcttgttgccaaaaggtcacagatatagacctgaagagttggttcacctttgggtggcagaaggatttgttggttcatgcaatttgagtaggagaacgttagaagaggttgggatggattacttcaatgatatggtctctgtatctttcttccaattggtttctcaaatgtattgtgattcgtactatgtcatgcatgatatccttcatgattttgcagagtcactctctagggaagactgctttagattagaagatgataatgtgacagaaataccatgcactgttcgacatctatctgttcatgttcaaagtatgcaaaagcataagcaaattatctgcaagctatatcatttacgcactattatctgcatcgatccgctaatggatggtccaagtgatatttttgatggcatgctacggaaccaaagaaaactgcgtgtattgtctctgtcattttacagcagcagcaagttgccagaatctattggtgagctgaagcacctccggtatttgaacctcgtcaggacgttagtttctgaattgcctacatcattatgtactctctaccacttacaattactttggttaaaccacatggtggagaatttgcctgacaaactatgcaatttaagaaagctacggcatctaggagcgtacgtgaatgatttcgcgattgaaaagcctatttgccaaattctgaatataggtaagttaacgtctctacaacacatttatgtcttttctgtacagaagaagcaaggctatgagttgcgacagttgaaggacttgaatgagcttggtggcagtttaaaagtgaaaaatcttgagaatgtcattggaaaggatgaagccgtagagtcgaagctatatctgaaaagtcgccttaaagagttggcatttgagtggagttccgagaatggcatggatgcaatggatattctagaaggtctaagaccgccaccccaactgagtaagctcagaatcaaaggttacagatctgatacatatcctgggtggttactagagcgatcctattttgagaatttggaaagttttgagcttagtaattgcagtttgctagaaggcctaccaccagatacagagctccttcggaattgctctaggttgcgtataaactttgttccaaatttgaaggaactatctaatcttccagcaggccttacagatttatcaattgattggtgcccactgcttatgtttatcaccaacaatgagctaggacagcatgacttgagggaaaatataataatcaaggcagacgacctggcatctaaacttacattgatgtgggaggtggattcaggaaaaaaagttaggagtatactgtcgaaagactattcatctctgaagcagttgatgacattgatgatggatgatgatatatcaaagcatcttcaaatcattgaaagtggtctggaggaaagagaagataaagtatggatgaaagaaaacatcatcaaggcatggctcttttgccatgagcagaggataagattcatttatggaaggaccatggagatgccattggttctaccgtcaggactctgtgaactttctctttcttcatgcagtattacagatgaagctttagctatttgccttggtggcctcacttcactgaggaatttaaaattgaaatataatatggcattaactacacttccatcagaaaaggtgtttgagcatttgacgaagcttgacaggttggttgtaataggttgtttgtgtctcaaatcactggggggcttacgtgctgctccatctctttcctgttttaactgttgggattgtccttctttagagctagcacggggagcagaactaatgccgttgaaccttgctagcaatctcagcatccttggctgcattcttgcagctgattcgttcattaatggcttgccacatctgaaacatctttccattgatgtctgcagatgctccccatccttatcgattggccacctgacctcccttgaatcattatgtctaaatggtctccctgatctttgctttgttgaaggcttgtcttccctgcaccttaagcgcctaagtttagtagatgttgcaaacctcactgccaagtgcatctcacagtttcgtgtccaggaatcgctcagggttagtagctctgtattgctcaaccacatgctaatggctgaagggtttacagccccaccaaatcttactcttttagattgcaaggagccgtcagtttcatttgaagaacctgcaaatctctcatccgtcaagcacctgcacttttcatgttgcgaaacagagtccctgcctagaaatctaaaatctgtctcaagtctggagagtctttctatagaacaatgccccaacatagcatctttaccagatctgccgtcctccctccagcgcataactatattgaattgccccgtcttgatgaagaattgccaagaacctgatggagaaagctggccaaagatttcgcacgttcgttggaagagctttccaccaaaatcgatctggcttccttag

SEQ ID NO: 2 - DNA, 1914 bp, Zea maize
atggcggagaggttgcctgacaaactttgcaatttaagtaagctacgacatctaagagtgaacaacaatcaaattcccaacattggcaagcttacttcattacaacgaatagagatattttccgtgcaaaagaagcaaggatatgagttgcaacaactgaagtacttgaatgagcttggtggcagtttaagcgtacaaaatcttgagaatgtcatcggaaaggatgaagccttagagtcgaagctatatctgaaaagtcgccttaaagagttgacacttgtgtggagttctgataatggcatggatgcaatggatattctgcatttggatattctagaaggtctgagaccgccaccccaattgagtaaactcacaatcgaaggctacaaatctagcacatatcctgggtggttacttgagcgatcctattttgagaatttagaaagttttgagctcaataattgcagtttgctagcagtcctaccaccagatacagagctccttcggcattgctctaggctgcatataaaaaatgttccaaaattgaaggaactaccgtatcttccagcaggccttacagagttgtcaatttgtaggtgtccattacttatgtttatcaccaacaaggagctaggacaacatgacttgagggaaaatataatgaaggcagacgacctgtcgtctaaacttgcatcgatgtgggaggtggattcaagatcacatgttacgagcgtactgtcggaagactattcatttctgaagcagttgatgacattgatgatggatgatgatatatcaaagcatcttcaaattattgaaagtggtctagaggaaggaggagatgaagtatggatgaaagaaaacatcatcaaggcatggctcttttgccatgagcagaggataagattcatttatggaaggaccatggagatgtcactggttctaccgtcaggactctataaactttctctttcttcatgcattattacagatgaagctttagctatttgcctcagtggcctcacttcactgagaactttggaattgaaatataatatgacattaactacacttccgtcagaagaggcgtttcaacaaatgacaaagctgaagtgcttcgctataagtggttgttggtgtctcaaatcactggggggattacatgctgctccatctctttcggctcttgattgttgggattgtccttctttagagctagcacgtggagccgaactaatgccattgaaccttgctagctaccttgacatccagggctgcattcttgcagccgattcattcactaattatgtgccagacctgaaacaacttaccattattaactgcagatgctccccatccttatcgattggccacctgacctcccttgaatcattacaactaattggtctccctgatctttactttgttgaaggcttgtcttccctgcaccttaagcgcctaaagttaggagatgttgcaaaccttactgccaagtgcttctcacagtttcgtgtcatggaatcgctcaccgttagtagctccgtattgctcaaccagatgctcatggctgaagggtttatggtcccaccaaatcttgaattcttatattgcaaggagccgtcgattttatttgaagagcctgcaaatctctcatctgtcaagtgcctgaatttttcgttatgtgaaaccgagtccctgccaagaaatctaaaatctctatcaagtctggagagtctcgagatagggttttgccccaacatagcatctttaccagatctgccgtcctccctcgagcgcataactatatgggagtgccctgtcttgaagaagaactgccaagaacctgatggagaaagctggccaaagatttcacgcatccgtcggaaggacataggcttccaatattttatttag

SEQ ID NO: 3 - DNA, 24 bp, Zea maize
gcatcttcaaattattgaaagtgg

SEQ ID NO: 4 - DNA, 24 bp, Zea maize
gcatcttcaaatcattgaaagtgg

SEQ ID NO: 5 - DNA, 23 bp, Zea maize
gatctgatacatatcctgggtgg

SEQ ID NO: 6 - DNA, 23 bp, Zea maize
aatctagcacatatcctgggtgg

SEQ ID NO: 7 - DNA, 23 bp, Zea maize
ccttctttagagctagcacgtgg

SEQ ID NO: 8 - DNA, 23 bp, Zea maize
ggctcttttgccatgagcagagg

SEQ ID NO: 9 - DNA, 23 bp, Zea maize
gctttagctatttgccttggtgg

SEQ ID NO: 10 - DNA, 3399 bp, Glycine max
ctcaataatcacttttatcatttcaaacaaagaaagttgttagtgcttaacattcctttgaatattaaactaagttcaatttttatttcttaccattagcgtgacatgaaaaaataaatttattaattccaatatatattggtggtataaagcacttccatatatgattggtcacaatttttttttacttagattccatcttcattgaaaaaagttaaaacacatgaaaaattaattatttcagttaaattaattcctttcactttttaaatatattctttatttgggtaaaataattcctttttgttatgtgtgagtttgaaattcttttaatttaatatatttgtaaataaattattttgacctaatatattgtaaatcaattcaaaaatagaatttactgtctaaagactcattattcaaccaaacgagagagttgtgttattctatagtgacggagcaacagaaaggttaagaatgtagcataaccaaaacaatgaaacaggtgatgtagaagatcatgctgtgaacggaggtagcaatggcgatgatgctttgactataaataagttgctatccgatctagcaaggcaagaagactactttgataaaagcttacagtggcgggagttccagggcaagaagcgcaagagacaagatgacaattggttggataaactaaaggacctgaaaaaaagagccattgatgtgaaaaactcactgcatcagtctgggtcgactaatgaattccccaagccttctgaattgggtgatgagtttttttatttatcgatagagaagcgttgggcgtcgcgagataaaaaagtggagaacatgtgggatcttctggaggatgaggaagtcttcattattggcatagatggaatggggggagttggaaaaacattcatggcaactcatatcaagaatgagattaaaagaaaggggactttcaaggatgtcttctgggtcactgtttcccatgatttcaccaatttcaaattgcaacatgacattgcagaaacaatacaggttaagctttacggagatgagatgactagagcaacaattttgacgtcagagttggagaaaagagaaaaagcactgcttattttggatgatgtttgggaatatattgatctgcaaaaggtggggattcctcttaaagtgaatggcattaaattgattatcacaactcgtttgaaacatgtgtgtctacagatggattgccaaccatataatataataacaatattcccctttgaagaagaagaagaagaagaagaagaagaagaagaagaagaaaaagaagaagaagaagaagcttgggagttatttttgctaaaacttggacaccgtggaacacctgcaagacttccccctcatgtactagagattgcaagatctgttgtaatgaaatgtgatggtttaccacttggaatcagtgtgatggctcgaaccatgaaagggaaaaatgagatccattggtggagacatgcattgaataaacttgacagattggaaatgggagaagaggtcttaagcgtactaaaacgtagctatgacaatttaattgaaaaggacatccaaaaatgtttcttacagtctgcactgtttcctaatgctgatgaagggaaatgggctatgatgattgttgagagtgggttgttaaatggaaaggggagtttggaggaaatatttgatgaggcacgtgtcatagtggataaactcataaaccattctttgttgttaggttattggagtttacgaatgaatggtctgttgaggaagatggcgtgcaatatcttgaacgagaatcacacttacatgataaaatgtcatgaaaatttgagaaagatacctcagatgcgggaatggacagctgatctggaggcagtttctttggcgggtaatgagatagaagaaatagcagagggcacatcacctaattgtccacgcttgtccaccttcatcttatctcgtaattccatcagtcatattcccaagtgttttttcagacacatgaacgctctaacacaacttgatttatcatataatcgtagattaacatctttgccaaagtcgctgtctaagttgaggtctcttacttctttagtgctccgccaatgttcaaaattgaaagatatacctccactgggagatctacaagcattgtcaagattggacatttccggttgtaattcgctcctcagggtaccggaaggcttgcaaaatctaaaaaagttgcaatggcttagtctttcccgcaagctgaatttatcattagtaccgttatgcgtactgcccggtttgagcaatatgcaatatctggatctccgcggttggtctggtataaaagtagaagatgtaaaagggatgactatgcttgaatgttttgcagtaagctttctcgatcaggattactacaaccgttctgtgcaagaaattcaggacactggttatggacctcaaacctattttatctattttggaaaatttaaggattacacacttggattttctgagaatcttatttatggtgaattcaagcatcgaagggtatgttttggagattgcgatggattacactatttactgccaagagaccttgcagaattacttgtaagtggcaatgatcaatgggaatgcttatgtgctcctctgtcatctaatggttctctatctttaaagcacattaccattcgggactgcacaaaattgaagagtttattctgtgtatcttgtcccttatgcactaatatccaaaacctcaaatctttgacacttaataatttggatagtttaagtgtcatctgcaaggaagatgttgctggtttaacacaatctttatctcggaggggggtgttttctcatctcaaggaattgagtatcagtggatgccatcaaatagagaagttgctgacgccagggttagtgccacaacttcaaaacctgaagtctatatcggtatcgaactgccaatcaataaaggagatatttgcaggagatagttcccacaacattgcacttcccaatttaaccaacttgcaactatactggttaccagacttaaagacagtgtgcaaaggaattttactcattaactctgaggatatattgcacatcaacaattgtcccaattatgaaaaacccagaattagtcgtgtatgattgattctgttgattcagattatggtacttattttatgtggcttagtctttgtattcgtaattcttgcaaagaaaaaacaaaatcataatttgctttttgaaatagtatactggcttttattggtaccattcataatcggttcggggaagaatgtatttccgggcattgcaatttcatatggtggagggaggtttggcaagtatccaacaactccctctctggtctcc

SEQ ID NO: 11 - DNA, 3800 bp, Glycine max
caaagtttgatttttattttaaaatcctcaattttatagtttgtgtgtgagagagaaagatttgccctatcaaacttttcttaattgttagcattattataagtaccctatcatctttaagatattaagttagtattaatagtattagtatgttactatttgacatattttttcttgattttggttaaagtttgaagatggtgactatgttttgttttgtctatatcttttgttgcattgaagcggctgaaggagacagtaaaatgattgttggtggttcagttaaccctcaaaacaatacacaattctcagctgctttattaggaggtacgcattctagttgccattccaatatattcttaaatcttaccctcaccaattccattatactattttccttcttcacacggatgagccttttatttttttatttaggtgatacaacacatagattttttttttaattctcaataatcagttttatcatttcacacaaaaaagttgttagtgcttaacattcctttgaatattaaactaagttcaatttttatttcttaccgttagcgtgacatgaaaaagtaaatttattacattccaatatatattggtgctataaagcactttcatatatatatatatatgaatggttacatttttttttttacttagattccaccttcattgaaaaaagttaaaacacatgaaaaattaattatttcagttaaattaattcctttcagtttttaaatatattctttatttgggtaaaataattctttttgttatgtgtgagtttgaaattcttttaatttaatatatttctaaataaattattttgacatataatatattgtaaatcaatttaaaaatagaattttctgtctaaagactcattattaaaacacacgagagagttgtgttattctacagtgaaggagcaacagaaaaaatttaagaatgtagcataaccaaaacaatgaaacaggtgatgtagaagatcatgctgtgaacggaggtagcaatggcgatgatgctttgactataaataatttgctatccgatctagcaagggaagaagactactttgataaagaattacagtggcgggagttccaggccattaagcgcaagagacaagatgacgattggtcggataaactaaaggacctgaaaaaaagagttattgatgtgaaaaactcactgcatcagtctgggtcgactaatgaattgcccaagccttctgaattgcatgctaagtttatttatttattgatagagaagctttgggagttgcgagatgaaaatgtgaagaagatgtgggatcttctggaggatgaggaagtcttcattattggcatagatggaatggggggagttggaaaaacattcatggcaactcatttcaagaatgagattaaaagaaaggggactttcaaggatgtcttctgggtcactgtttcccatgatttcaccattttcaaattgcaacatcacattgcagaaacaatgcaggttaagctttacggagatgagatgaccagagcaacaattttgacgtcagagttggagaaaagagaaaaaacactgcttattttggatgatgtttgggaatatattgatctgcaaaaggtggggattcctcttaaagtgaatggcattaaattgattatcacaactcgtttgaaacatgtgtggctacagatggattgcctaccaaataatacaataacaatattcccctttgatgaactagaagaagaagcttgggagttatttttgctaaaacttggacaccgtggaacacctgcaagacttccccctcatgtactagagattgcaagatctgttgtaatgaaatgtgatggtttaccacttggaatcagtgcgatggctcgaaccatgaaagggaaaaatgagatccattggtggagacatgcattgaataaacttgacagattggaaatgggagaagaggtcttaagcgtactaaaacgtagctatgacaatttaattgaaaaggacatccaaaaatgtttcttacagtctgcactgtttcctaatcatatttttaaagaggaatgggttatgatgcttgttgagagtgggttgttagatggaaagaggagtttggaggaaacatttgatgagggacgtgtcataatggataaactcattaaccattctttgttgttaggttgtttgatgttacgaatgaatggtctggtgaggaagatggcgtgccatatcttgaacgacaatcacacttacttgataaaatgtaatgaaaaattgagaaagatgcctcagatgcgggaatggacagctgatctggaggcagtttctttggcgggtaatgagatagaagaaatagcagagggcacatcacctaattgtccacgcttgtccaccttcatcttatctcgtaattccatcagtcatattcccaagtgttttttcagacgcatgaacgctctaacacaacttgatttatcatttaatcttagattaacatctttgccaaagtcgctgtctaagttgaggtctcttacttctttagtgctccgtcaatgttcaaaattgaaagatatacctccactgggagatctacaagcattgtcaagattggacatttcaggttgtgattcgctcctcagggtaccggaaggcttgcaaaatctaaaaaagttgcaatgccttaatctttcccgcgatttgtatttatcattgttacccggatgcgcactgcccggtttgagcaatatgcaatatctggatctccggggttcgtcaggtataaaagtagaagatgtaaaagggatgactatgcttgaatgttttgcagtaagctttctcgatcaggattactacaaccgttatgtgcaagaaattcaggacactggttatggacctcaaatctattttatctattttggaaaatttgatgattacacacttggatttcctgagaatcctatttatctttgtcttgaattcaagcgtcgaagggtatgttttggagattgcgatgaattaccctatttactgccaagagaccttacggaattacttgtaagtggcaatgatcaatgggaatgcttatgtgctcctctgtcatctaatggtcctctatctttaaaggacattaacattaaacactgtacaaaattgaagagtttattctgtgtatcttgttccttatgcactaatatccaaaacctcaaatctttgaaacttgataatttgggtagtttaagtgtcctctgcaaggaagatgttgctggtttaacacaatctttatctcggagtggggtgttttctcatctcaaggaattgagtatcgagaaatgccatcagatagagaagttgctgacgccagggttagtgccacaacttcaaaacctggcgtctatatcggtagaggactgcgaatcaataaaggagatatttgcgggagatagttccgacaacattgcacttcccaatttaaccaaattgcaactacgctatttaccagaattacagacagtgtgcaaaggaattttactctgtaactctgagtatatattctacatcaaggattgtcccaattatgaaacacccagaattggtggtcgtgtatgattgattctgttgattcagattatggtacttattttatgtggcttactctttgtattcgtaattcttgtaaagaaaaaacaaaatcataatttgctttttgaaatagtatactcgcttttattggtaccattcatagtcggttcggggaagaatgtatttccgggcattgcaatttcata

SEQ ID NO: 12 - DNA, 23 bp, Glycine max
gtgggatcttctggaggatgagg

SEQ ID NO: 13 - DNA, 23 bp, Glycine max
gtgggttgttaaatggaaagggg

SEQ ID NO: 14 - DNA, 23 bp, Glycine max
gtgggttgttagatggaaagagg

SEQ ID NO: 15 - DNA, 23 bp, Glycine max
ggaatggacagctgatctggagg

SEQ ID NO: 16 - DNA, 23 bp, Glycine max
gcttgtagatctcccagtggagg

SEQ ID NO: 17 - DNA, 23 bp, Glycine max
aaatagataaaataggtttgagg

SEQ ID NO: 18 - DNA, 23 bp, Glycine max
aaatagataaaatagatttgagg

SEQ ID NO: 19 - DNA, 3135 bp, Glycine max
atgggtggggttggaaaaactactttggcccaattggtgtacaatgatgagaatttgaaacagatatttgattttgattttaaggcatgggtttgtgtttctcaagaatttgatgttctcaaggtcacaaaaactataatagaggcggtgactggaaaggcttgtaaattgagtgatctgaatctacttcatcttgaattgatggacaagctgaaagataaaaaattcttaattgttttggatgatgtttggacagaggattatgttgattggcgtcttcttaagaaaccatttaaccgtgggattattaggagaagtaaaattcttctaacaacccgcagtgaaaaaacagcatctgtagtccaaactgttcacacctatcatctaaaccaattgtcgaatgaagattgttggtcagtgtttgcgaaccatgcatgtctttccacggaatctaacgagaacacagcaacactagaaaaaattggaaaggagattgttaaaaagtgcaacggactgcctttagcagcagagtcgcttggaggcatgttgagaagaaagcatgacattggggattggaataatattctcaatagtgacatttgggaactttctgaaagtgagtgtaaagttattccagcactgagacttagttatcattatctccctccacatttaaaacgatgctttgtttattgttcgttgtatccacaagattacgaatttgaaaaaaatgaattaatcttgttgtggatggctgaagatcttttgaagaaaccaaggaaaggtaggactttagaagaggttggtcatgagtattttgatgatttggtttcgagatcatttttccaacgttcaaacacaagtagaagtagttggccttatggcaaatgttttgtgatgcatgacctcatgcatgatctagccacatcactcggtggagatttttactttagatcagaagaacttgggaaagaaacaaagatcaacaccaagactcgtcatttgtcatttgccaaattcaattcttcagtcttggacaactttgatgttgttggtagagcaaaatttctgagaactttcttgtccattataaattttgaagctgctccattcaacaatgaggaggcacaatgtatcataatgtcgaagcttatgtacttgagagttttatcattttgtgacttccaaagtctggattctttgcctgactcaataggtaaattgatccatctgcgctatttagatctctctttttcaagtgtagaaacactgccaaagtcattatgtaatttatacaatctgcaaactttgaagttgtgtagttgcagaaagctgactaagttgcctagtgacatgtgcaatcttgttaacttgcgtcatcttgagatacttggaactcctataaaagagatgccgagaggaatgagtaaattaaatcatttacaacatctggatttctttgctgtgggcaagcacgaagagaatggaatcaaagaattgggagcactttcaaatcttcgtggtcaacttgaaattaggaacttggagaatgtttcccaaagtgatgaagcgttggaggcaaggatgatggataaaaaacacattaatagtttacagttggaatggtctggatgtaacaacaacagtaccaacttccaacttgaaatagatgtgctttgcaagttacagcctcactttaacattgaatcgttgtatataaaaggctataaaggaaccagatttccagattggatgggaaattcttcctactgcaatatgatgagtctaaaattgcgtgattgtgacaactgtagtatgcttccttcacttggacaactaccttctctcaaggtccttaagattgcacgattgaataggctgaagactattgatgcaggtttttacaagaacgaagattgtcgttctgggacgccctttccctcccttgaatctctggccattcatcacatgccttgttgggaggtgtggagttccttcgattcagaagcttttcctgtgcttgaaattcttgaaatacgtgactgccccaaactagagggaagtttgccgaatcaccttcctgctctgaaaacacttacaattagaaattgtgagctgcttggctcttctctcccaacggctcccgccattcaaagtttggagataagtaaaagcaataaagtagcactgcatgcgtttcctctcttgctagagactatagaagtagaaggaagcccaatggtggagtccatgatggaggccatcacaaacatccaaccaacttgtctccggtctttaacattaagggattgctcgtcagccatgtcatttccgggtggtcgtttacctgaatcactgaagagtctgtatatcgaggatcttaaaaaactggaattcccgacgcaacacaaacatgagttactggaaacactgtcaatagaaagcagttgtgattcactcacatctcttccattggttacctttccaaatctcagagatgtcacaatcggaaagtgtgaaaatatggaatatcttttggtttcaggggcagagtcatttaagagtctgtgttctttgagtatttaccaatgccccaactttgtatcattcgggagagaaggattgcctgaagagatgagtactcttctcccaaagttagaagatctttacatatccaactgcccagaaattgagtcctttccaaaacggggtatgccacctaacctgagaacagtttggattgtgaattgtgagaaactactgagcggcctagcatggccatccatgggcatgcttactcatctcaatgttgggggtcgatgtgatggcatcaagtccttccctaaagagggtttgctgcctccctcccttacgtctctgtatctatttaagttttcaaatctggagatgttggactgcacagggcttctccatctcacatccctgcaagaattaaccatgaggggatgtcctttgctggagaatatggctggagaaaggcttcctgactctctaataaaattaaccatatgggaatgtcctttgctggaaaaacgatgccgcatgaagcaccctcaaatttggcctaaaatttcccacatccctggcattaaggttgacgatagatggatttag

SEQ ID NO: 20 - DNA, 3399 bp, Glycine max
atggctgaggcagttggtggtgcattcctctctgctttccttgatgttgtgttcgacaagctgtctacagatgaggttgttgacttcatccgtggaaagaagcttgacctcaatttgcttgaggacttgaagaccactctgagagtggttggagctgtgcttgatgatgctgagaagaaacaaatcaaactctccagtgtccaccagtggctcatcgaactcaaagatgctctctatgatgccgatgacttgctggatgaaatttctaccaaatctgcaactcgaaagaaggtatgtaaagtgctttctcgctttactgataggaaaatggccagtaagttggaaaaaatagttgacaaattagataaagttttaggaggcatgaagggtcttcctttgcaagtgatggcaggggagatgaacgagtcatggaatactcagccaacgacatcactggaagatggatatggcatgtatggtagggatacagacaaggaggccataatgaagttgttgttgtcagatgatagcagtgatggtgtactagtgtctgtgatcgctattgtaggcatgggtggggttggaaaaaccactttagcccgttctgtgttcaacaatgagaatttgaagcagatgtttgatttaaatgcatgggtttgtgtttctgatcaatttgatattgttaaggtcacaaaaactatgatagagcaaatcacgcaagagtcatgtaaattgaatgatctaaacttgcttcaacttgaattgatggacaaactgaaagttaaaaaattcttaattgtcttggatgatgtatggatcgaggattatgagaattggagtaatcttacaaaaccatttctacatggaaaaaggggaaattgttggctagtgtttgcaaaccatgcatttccccccttagaatcaagtggggaggatagaagagctttagaagaaattggaagggagattgttaaaaagtgtaatggattgcctttagcagcacggtcacttggaggtatgttgagaagaaagcatgctattagggattggaataatatacttgaaagtgacatttgggaacttcctgaaagtcagtgtaaaattattccagccctgagaattagttatcaatatctccctccacatttaaaacggtgctttgtttattgttcattataccctaaagattatgaatttcgaaagaaggacttgatcttgttgtggatggctgaagatcttttgaagcttccaaacagaggaaaggcattagaagttggttatgagtattttgatgatttagtttcgagatcattttttcaacgttcaagtaatcaaacttggggcaattattttgtaatgcatgacctcgtgcatgatctagcattataccttggtggagaattctatttcagatcagaagaacttggaaaagaaaccaagattggtataaagactcgtcatttgtcagttacagagttcagtgatccaatctcagatattgaagtttttgacagactacaatatttgagaactttattggcaattgattttaaagattcttcattcaacaaggaaaaggcaccaggtaaattgatccatttgcgttatttaaatctctctcatacaagtataaaaacactgccggagtcattgtgtaatttgtacaatctacaaactctggcgttgtctcgttgcgaaatgttgaccaggttgcctactgacatgcaaaatcttgtaaacttgtgtcatcttcatattgatcatactccgataggagagatgcctagaggaatgggaatgttaagtcatttgcagcatttggatttctttattgtgggcaagcataaagagaacggaatcaaagaactggggacactttcaaatcttcatggttcgctttctattaggaatttggagaatgtaaccagaagcaatgaagcattggaggctaggatgatggataagaagaacattaatcatttatcgttgaaatggtctaatggcaccgacttccaaactgaattagatgtactgtgcaaattaaaacctcacccaggcctggaatctctatcgatatcgggttataatggaaccatatttccagagtgggtgggaaatttttcctaccacaacatgacaagtctaagtttacgtggttgtaataactgttgtgtgcttccttcgcttgggcaactaccatctcttaagcagctctatatttcaagattgaagtcagtgaagactgttgatgcagggttttacaaaaatgaagattgtccttcttctgtgacacccttttcttcccttgaaacgctatacattggtcacatgtgttgctgggagttgtggagtatccctgagtcagacgcctttcctctactcaagtctcttacaatagaggattgccccaaactaaggggagatttgccaaatcaccttcctgctctggaaacactcaatattacaagatgccagcttcttgtctcttccctcccaagggctcccacccttaacatattagtgatatggaaaagtaacaatgtatcgttgcatgtgtttcctcttttgttggaatggatagatgtagaaggaagcccaatggtggagtccatgatcgaggccatctccagcatcgagccaacttgcctccaacgtttaagattgagggattgttcgtcagccatatcttttccgggtggtcgtctacctgcatctctgaaggatctgcatatcagcaatcttaaaaatctggaattcccgacccaacacaaacacgatttactggaatcactgtcactatacaatagttgtgattctctcacgtctcttgcattggctacctttccaaatctcaaaagtctcggaatcgataactgtgaacatatggaatctcttttggtttcaggggcagagtcatttaagatctttctccaaatatccaactgcccagaaattgagtcgtttccagaagggggtatgccacctaacctgagaacagtttcgattgagaattgtgagaaactaatgagcggcctagcatggctatccatgggcatgcttactgatctcactgtttggggtcgatgtgatggcatcaagtcattccctaaggagggtttgctgcctccctcccttacgtttctgtatctatatggattctcaaatctggagatgttggactgcacggggcttctccatctcacatccctgcaagaattaaccataagggaatgtcctttgctggagaatatggtgggagaaaggcttcctgtctctctaataaaattaaccataagcggatgtcctttgctggaaaaacaatgccgcaggaagcaccctcaaatttggcctaaaatatcccacatccgtcacattaaagttgacagtagattgatttag

SEQ ID NO: 21 - DNA, 23 bp, Glycine max
gatctagccacatcactcggtgg

SEQ ID NO: 22 - DNA, 23 bp, Glycine max
gatctagcattataccttggtgg

SEQ ID NO: 23 - DNA, 23 bp, Glycine max
ccaaagtgatgaagcgttggagg

SEQ ID NO: 24 - DNA, 23 bp, Glycine max
cagaagcaatgaagcattggagg

SEQ ID NO: 25 - DNA, 23 bp, Glycine max
ggaatatcttttggtttcagggg

SEQ ID NO: 26 - DNA, 23 bp, Glycine max
ggaatctcttttggtttcagggg

SEQ ID NO: 27 - DNA, 23 bp, Glycine max
attgagtcctttccaaaacgggg

SEQ ID NO: 28 - DNA, 23 bp, Glycine max
attgagtcgtttccagaaggggg

SEQ ID NO: 29 - DNA, 23 bp, Glycine max
tggagatgttggactgcacaggg

SEQ ID NO: 30 - DNA, 24 bp, Glycine max
ctggagatgttggactgcacgggg

SEQ ID NO: 31 - DNA, 23 bp, Glycine max
gcaaacttccctctagtttgggg

SEQ ID NO: 32 - DNA, 23 bp, Glycine max
gcaaatctccccttagtttgggg

SEQ ID NO: 33 - DNA, 21 bp, Artificial Sequence
  Synthetic
atgagtattttgatgatttgg

SEQ ID NO: 34 - DNA, 24 bp, Artificial sequence
  Synthetic
ggttacgagtattttgatgattta

SEQ ID NO: 35 - DNA, 22 bp, Artificial sequence
  Synthetic
cattatgatacattgtgcctcc

SEQ ID NO: 36 - DNA, 20 bp, Artificial sequence
  Synthetic
ctacaatacctggtgccttt

SEQ ID NO: 37 - DNA, 21 bp, Artificial sequence
  Synthetic
attacaatacctggtgctttt

SEQ ID NO: 38 - DNA, 22 bp, Artificial sequence
  Synthetic
atggaatcaaagaattgggagc

SEQ ID NO: 39 - DNA, 22 bp, Artificial sequence
  Synthetic
atggaatcaaagaattgggagg

SEQ ID NO: 40 - DNA, 22 bp, Artificial sequence
  Synthetic
acggaatcaaagaactggggac

SEQ ID NO: 41 - DNA, 23 bp, Artificial sequence
  Synthetic
agtgaggctgtaacttgcaaagc

SEQ ID NO: 42 - DNA, 22 bp, Artificial sequence
  Synthetic
acwaacatccaaccaacttgtc

SEQ ID NO: 43 - DNA, 22 bp, Artificial sequence
  Synthetic
ctccagcatcgagccaacttgc

SEQ ID NO: 44 - DNA, 22 bp, Artificial sequence
  Synthetic
cttcagcattgatccaacttgc

SEQ ID NO: 45 - DNA, 22 bp, Artificial sequence
  Synthetic
ttgggagaagastactcatctc

SEQ ID NO: 46 - DNA, 21 bp, Artificial sequence
  Synthetic
tccagcaaaggacatcccctc

SEQ ID NO: 47 - DNA, 20 bp, Artificial sequence
  Synthetic
cgtcaaccttaatgccaggg

SEQ ID NO: 48 - DNA, 21 bp, Artificial sequence
  Synthetic
agatgcagagacgtaagggag

SEQ ID NO: 49 - DNA, 21 bp, Artificial sequence
  Synthetic
attagagagacaggaagcctg

SEQ ID NO: 50 - DNA, 21 bp, Artificial sequence
  Synthetic
acatcccattatggttaattg

SEQ ID NO: 51 - DNA, 21 bp, Artificial sequence
  Synthetic
tttccagcaaaggacattcca

SEQ ID NO: 52 - DNA, 21 bp, Artificial sequence
  Synthetic
tccccttatggttaattttac

SEQ ID NO: 53 - DNA, 22 bp, Artificial sequence
  Synthetic
aggaagactttctccagccatt

SEQ ID NO: 54 - DNA, 21 bp, Artificial sequence
  Synthetic
cccaaatgccagggatgtggc

SEQ ID NO: 55 - DNA, 20 bp, Artificial sequence
  Synthetic
tttgagggtgcttcatgcag

SEQ ID NO: 56 - DNA, 20 bp, Artificial sequence
  Synthetic
tgacggatgtgggatatttg

SEQ ID NO: 57 - DNA, 20 bp, Artificial sequence
  Synthetic
tttccagcaaaggacatccg

SEQ ID NO: 58 - DNA, 20 bp, Artificial sequence
  Synthetic
tctccagcaaaggacatcta

SEQ ID NO: 59 - DNA, 20 bp, Artificial sequence
  Synthetic
caaaggacatctctctatga

SEQ ID NO: 60 - DNA, 20 bp, Artificial sequence
  Synthetic
aagcctttctccagccatac

SEQ ID NO: 61 - DNA, 20 bp, Artificial sequence
  Synthetic
ggaaaggcttgtaaattgag

SEQ ID NO: 62 - DNA, 22 bp, Artificial sequence
  Synthetic
acagaggattatgttgattggc

SEQ ID NO: 63 - DNA, 20 bp, Artificial sequence
  Synthetic
ggcatgggtttgtatttcta

SEQ ID NO: 64 - DNA, 22 bp, Artificial sequence
  Synthetic
gatattctgaaggtcacaaaag

SEQ ID NO: 65 - DNA, 20 bp, Artificial sequence
  Synthetic
aatagaggcggttactggac

SEQ ID NO: 66 - DNA, 20 bp, Artificial sequence
  Synthetic
acaagctgaaagataaaaag

SEQ ID NO: 67 - DNA, 20 bp, Artificial sequence
  Synthetic
gaattgatggacaagctaag

SEQ ID NO: 68 - DNA, 31243 bp, Glycine max
ttttctcttgaactgataatcaaatagttattgagatttttaattgagctgcatttgttaagaagtcacggctaaaagagttacctagttgtcagttatactattttcatgactaagcagcaagcacagatattgcagtgatacacaaccgagagcatattctccaaaaggcaaattgccttgatgcaatttgctagtttgtacactgatagaattgcttatttatcaatagtgttccaatgtataggtatctcatggcactgattaaggataaaacatggtgatttattcctttctaaaatcttttgtccctgcacaagttgtttatattaaacattgtttaccttacttttgctcacaagatgaaagaaggaagaagatagttgagatgggtggagctcaagaactcttaaatatgttaagcactgctaaagacgaccgtacacggaaagaagcattgcatgctcttgatgcactgtcacaatcaggtgaaatcataattttaatatttttttaaatagttattatcatgctggtggagaggtagattattgtgatcaattagtacctttgtggttctaaatagtaaaccagaaatgcccaaccacttatggaatttgttaatttatttgtataatattgagctggaaatcaattttatgagcaaagtgtgataagaagcatatgaaacttttatatgtttccagtttctgttatccttattcaatagatatgggcttgtaaagatgaaaatgaacataaattgttttgtgcattaattttgggacatattatacgtgcacaagcttatgtgtaacaatatctatacctgctactttccctgtcaacatattgatttttaagaatccagttcaagtaatatttatgaggttgaaagatatgcaacagtacaaccaaattagtagtgctagctagtactagccttttctgttctctttcgattgagataagctacttcaatgttatagatgaagctcttgcatccttgcatcatgctggggccatttcagtaattaggtctgcaccaaattcacttgaggatgcagaagttgagggattcaagttgagcttgatgaaaagatttcaagatctcagatatgatgtgccatcatgacttgaggtgcatgcctccttttgctttatgtttttggttggttggagcatgaaataacatgatatgagaaattaagctggcaaccaaagcttttgtggggaagagtacttgaaattactgtgtatcatttgaccaaatctaatggaagattatagttctattgtcattttagtttttttcacttgtcaaatgcgatttgtcgctcattgttctgtcaatcataataaaatggaaaagatttatgtgcatgtcaatttttattttttgaaatatgtgtttagaagataaaagattacaacaaactagtattgaagttgtaagtgtttagatactgtaattgtatatttggttaacactactagattaaatttaagcctcaactttcaaatgtgattgatcatataatgtcataaaatgtgtgtaattataggttgatgctttaattgttatttacatatgcctcaactctcaaccgtatgtcatcatcaggcttcttgtttaggttcagctggcgccttgctcgttctattttgttcgtattcctttgttcattcgatgtttttttaggaaaatatgttcgttgaaagaaaaaatcagtcaacagaagatacatgcccttacttttctctactccacgtctccacctaccctaacccttggagttacttttcaattgagcacgttaacaagcctaactaaacgtggttctgtggagataatatactaaaaaaatattattttttatttaatttaataagacttgtgcgcgtaactcttttcaaagtgctagctttcttttttggtgaattttcaaagtgctaggtgaatatgcgtatttggagatagaaagcttttttttttgggacacaaaagcttgtttaacatgtgataaacttaaaactaataatcattttttttaattatccctattcaatgttttagttttaaaaataccccatttgggaaaatagcccatctgtggatgtaaaaattactagagtacaagttaattagggttagttgttttttttttctttcttcttttcctacgagatcaagaggaacggagcaaaatcatgttttttcttccaccaaaataatgtaaaattttaaaacaaaatactaaaataataggttataatatatttcttttccttcattttatacttagtcttttattttttttaaaaatatcattctagttatttaactctcacatttgagttaatgttatacttttgaaacttcagtcattttttatttattttggatacgattttgagccttttttcttttactaattaaagatataaaatttgtctcattaaattaaactatgaatccaattaatgttcaaacaaaacataaatccttaacatgatgaaaattgaatgaaaaatgaatttcataagcaattggaaaactgaaaaaaaaaatctaataacaatatttgaaaatctattaacaatgagcagtaggcttctttggaacttgaaatgaagaataaaagagtcattggaaataaatctcaattaattgaaagatattttttagaaaatgtcattaaatagaataaaaataatcaaaatttgcttatatttgaatctaataaaaaaattgttaattactctttttgtctcgaatataaacaaaaaatactttgagtattagtctcaaataaaagtaaaatttaactattgttactttatttaatgagatattcctaaattatattttatttaattaaagttttattacttattatctctcttttttatttttgatatgaactttcaagaaagtgtagtttagaagaagaattttttttaataagaaaggtgtaattaaataatctaattatctaactactaactttttgaataaaccgtaagttaatttcttttatatagaaagaagggattaaattaattttaaaagagttcctcttcattttaatcattaatttttttgaaattcaataatcaatacctactcattacaataataaaatacaaaaacttcttcacgaaataaattgattccttgtgttatatatatatatatatatatatatatatatatatatatatatatatatatatatatatatatatatatatattcagtatataatttagtgtagctggacacatattagtgccccgtggccgtgtgttgtgcttttttgttgggcgaaacaacggccaaagcgacgaatcacttccttacgtgacacacctctgtctaatagacgataggccaaagtcacaaatactttttgattgagtattttttaatgccacatatcatatctgtcagcgtcacatgttcaaataaatccctagtaaaaacgccagaaaacaaatgcatgagcaatttttggactttggactagttacaatttttcaacgtcacatctttaaatgatttcgtctctatttagtagttgtttttaatgcggccatgcccactttctcgttacaaagcatgcattttattatttgaacgaaaatatttaatattgtgtattactcgttttacacaattgcttttattcttttttttttattttttaaatacagtcatctttaaaaacaaaatcttcgatcattccatttcattgttcacaaaacattatcctatcacatgcaccctatgtaatataatacacggttgtggataaaataattctgcacctgcccaacttttgtattgatatcatttttttatttcctctatattttccatatttatatattaattctatcactttcctgcaccccaataagtcatgctccaaatattattgttttggataagtatattgcacaatctattcttggcttcttcatgaccatgacacggcaatggagacgaacgataatgaaaggcgcgtaaatcatttgaaaggttgaattatgtaccaaatgctattatattagcatttcatacgccattctaacaataatgagaacgagttgccccacaattgatcaatatttgtatccttgcacggcacaaacttgtaagatatggccccaacttcgtcaccccatcaagttgatttcatttctttaatatttggtattttacatagaaatgctgccacaagacatgaattctacaataaacaacaagggatccaaaatacaaaagtaacacaatcgccacagcaaccaaatgcctctagaatctccccagccataccctctctccccaaataaaattttctatacatataaaaaaaacaatagaaggggagaaatgagagaaccagcttgtatttatgacttgctactaaaagcattatatatgttggtggaaatggcaagcacacttgtaaccacagctagtataatcattatcagtgcaataattttgtctcttctcgttgatatacctttaacatccctgtcatcagaaacaatgaaaattaagagactaatttatttatttattcaattcaattttcaacttgagctctactttatcagaagtcaataagtctatgctagattaccttaaaacaatagagccggggaaaatgaaggcaaggcacactgcggatgaggatcccaggaactgaaagaagtaccaaatatctgggattgctatagctgcaaggtaggagaatacaagcagcaccagagtgaggatcataaatcttttgttgtctgtggctagcataggcttcttagggaagagaacttcatctatgttggttctcaaagagaagttcaagagaggaaacaccagcatgatgtggagggcatagcttacacggaccaaactattgagcaaggaaccaactgctgaaccagcattctggtcaaaattgatgagaatgtctgactgggttgaatccccaaataacatgtacccaaataagcctattgcaaggtagatcacagcacaaagcaataatgctaatcgaactgctgttgtcatttgggatgccttggcaagctcaaacccaatggggtgcactgaaagtaaaatcaaccatcagcacagaaattttctaggcatacccttaaaaaaaatgagcaaatccattaggccaattaccattaaagtgaaatgtgaaggctgtgacaacaacaggaactgcagtgaacagatcaaagaatgaggtttggtagtctagccgaggaaacaatctaggagtttgtgtttttccttgcaccagagctgtgatagccaacccacaacatatgccaacaaatgccactgcaagaagagttgacactgcagagctgtacttcaaggactctaccaattccaaaacaccaagaggaagaacccatgttagttactgaaactcttcaattccaaatacacaagaaagcatgttatataacaaaatattcaattgtaacactcacctacacgtttgtacaataccaatggaagcataacaaagaccaaggtgaaaagcaaagcaaattcccgggaattccaccagtgaattccaaaccactgttgcaaaatgcccaaatgcacttcccctccattttgctttccagatagcacatctcctgttgttcaacaaaaggtaattattaaaatacatctatttttttctttcatcttctttctactacattttcttcttatatttctctttatttcctgtcatttcacttttttttttcctgtctttcttctacccattacatagaccaaaaattgaggtgtgcattgcggaaacagattccccacattcactttttttttcatgaatcagaactattagattgaatatcgaaggttatatttggaatacatattttaagagtatgtttggatacaaagttagaagtgcatttgacaacttttgggagctcctctaatggaaaaagattaatatttttagtagaaaactctcaaaaacacttctagtttgtatcgaaacaggcctaagttagattcattgagataagttatgagtaatacaatctgtatttaacagtgaattcccagcggtaggaaatcccgatccttacatttccattatcttgttaaattaattaccatacacaaacattaaagaaaacgacttactacatatattttttcaaaaaatgaacctttctatttatagtaaaaaaaataaaaaacaaatttcacttattattagcaacaatttcaccaatcaaaatgaatctgactgaaaacccggcaaaactcagaacaagcataccaaaccaaaaacatgaaaaaatctacatttttttttccttttttacgaattcagtagaaaggaaattaaaaaaaaagggaaaagttccgttacgttaccgatgatgataaggtagagaattaaacccccaacgttggtgatgatgacgcaaacttgcgcggctaatgctccacccgatccgaacgcctccctcatgacgccagcgtacgtcgtcgtttcgccggagtgcgtgaaccgcatcaggaagtccacggacagttccgccagcacggccaccacgagaatcatcgcgaaagcgggaactacgccgagaaccttcatgatcgccggaatcgacatgattccggcgccgactatgctggtggccacgttgaacaccgcgccggggacggaagccggcggcggcgttcctttggaatcccccaggagggggacgctgactccggcggccggagacatgccggaggcaaaattgtgaggatcggagaaagtgcggtggcggtgtgcggtgcctggcagcctactatctttgaattgaatggtttttgttttgttgtctctcacgaaaatttcacttcctctctctttataaatgatacaagtggatttgggaagttaagaaaacaaaaaatgaagttataataagtaagattttattttataagttttgtaggatgaaaagaaatatagttgaatgaggaaatttcattgaaaatagttagctagattttataatagagattaaacaataataaaatctgcagatacttcaacatgagtatgataataataataataaaaaattgttgttttctatttttactccaacatggactgaaattcatatgaatttttttgaatagtctatttttttttatttaatttaatattcatatcaaagttatttcatactgaaaaaaatattaaatactagcattctattattaccatttggaggaatgattgaaagagtgttaaagtgcaccttttcagtcaacagttaaaaataaggcgtttaattcaattcaatattacaaagttaagttggctgtataataataacagtggtagtaagtagtagagtgaaagaaaaatttttttggtcaaaatatttaaatcaagactagaagatatgcaaatcagagattacattggatgatacggtcgaccaataaaaaataaaagaaaaaacataaattgggatgttcaaatactaataataataactctaaacaaacattaacacgtgagttttctttcccacgttgtaatcattttgaatttttaaaatgttatgacacaaataataagttaataataattataatttaacatttgaattgataaaagtgtttagttttattgtagattaaactaatctttcttcgagtaaaaataacattaaattcctacacaacaggtttatcagtttatagagtaataacactcttattcttaatcgttttcttttctggaagaaaaaataaatcttagtcttgttatttttttgagaatgtaaaatataccttaaaaaattcccttaaagtttgtataattttttggtatgtaaatatatttataaataaaaaaatgtttgcgaaaagtaatatttacataacaaacactatttacagaacattgatgaaattatttttagatatataattattaatacgaatatatgaatatgttattaaagtaatcaatagttatgttaaaactgatctgttgactagacagtttgtcaatttattttttattcacttaattgctatttttttctaggtttgttctttcgttaaaaaaccttgcattggaggaaggccaatgctagttataaaaatataaaccatgatttgaatataaaattatttttagtcgaaaaacaatgaattatgttgcaagtatcactattgaaaaaatgccaacggagcccaagaaggtgaggcccaaactgaaagcgtgaagcggcccaagactgagtgaggaaataaataattatccagaaaatcggaaatggacaatccttcttgttacgcaattctgaatttgcgggttttggatttggacttggtcgtcaacacagtctaattaatatctttttgctccttcgcttatgaatcttcttcttcttcttcttgttcctgcaacgcactgaattcgatcaatcaatccatcttcaattgctttgtttcgatcggaggaaaatggccgatcagttatcgaagggagaggaattcgagaaaaaggctgagaagaagctcagcggttggggcttgtttggctccaagtatgaagatgccgccgatctcttcgataaagccgccaattgcttcaagctcgccaaatcatgtttttcctctttctctctactttttttaaattccatttcgtgtctcctcaaaatgctgatttagtgtcataaatcataattattattctcttctattgttgttattttattgttattacttcaatcgacgagtgtgttgagttttgaggtgtccgatttcccgattaattgaagtatagttttaatctgattttactggaaaatattttttgcctgattttttttttttggaacaattactagcatataaattagaattgtggatgaagtacgacaatcaactctgtgttgtttgtgactgcgctcactttcaatttgacgactaatctctttattttgttgaaagtgacgaactttgaaattgatgttggaatagttctgtttattgttcttgatttgatctatgtggcattttaggggacaaggctggagcgacatacctgaagttggcaagttgtcatttgaaggtaacattcatcagacttggggttttggagtgggctgaatctcttttgcatcctttagttctctattaagcctgcatgacattgttgtgttctgtttccatttagttggaaagcaagcatgaagctgcacaggcccatgtcgatgctgcacattgctacaaaaagactaatataaacggtatgcatgtgtctcagttgttaccactacatgcactacaatactttctcatttatgatttgtgctttaaatgctgctcttgcttccatgcagcaaggccaattccttttagcctcaatgtttctctgtataactttaatgtaaatcatataaaacaattgctacctttttgcatgaacaaattatataaagcaaatctctttgtttaatctttacatatgtgtaaatcaaatactgggcttcatatcgataaggtctaagtaggggttcagtcttttatttggattagtttaagtcagaaattgaagttaatttgtgcttgcataagttgcttccatctgattgctttctttttatggctgtctgtatgtcatagccttattttgatttgttatttgctgactattattagattggaactcatgatcatatccctaagcaggagcaaattattttgctgtcttgcttgtcttagtatgtcccacttgcattaggaagaactaagacaattaaagttaccttttctttctttgaatacagagtctgtatcttgcttagaccgagctgtaaatcttttctgtgacattggaagactctctatggctgctagatatttaaaggtatattatgtttatgatattgatatctcttctcctgggtatgatttttaatttattctcttgtccatatcccagattttagatattgatcctgcaataaaatgcgttgaagtatactaagttatctgaatccccattaacatgttttaactgggttcactattttatacacaggaaattgctgaattgtacgagggtgaacagaatattgagcaggctcttgtttactatgaaaaatcagctgatttttttcaaaatgaagaagtgacaacttctgcgaaccaatgcaaacaaaaagttgcccagtttgctgctcagctagaacagtaagatattgtcctttctgcatatattatctcttttattatgctgatgaattgatcaatatttcttcaacttgggtttattctttaattggttagtaatttcttctgagaactttctttctggcctttattttgttcagtaccctttctctaacccactctcctcaggttaacattagcttaggtcagtgtaggttgtttgacactgagtttttattggtatggatgtatggtctattatgatctcaatggaaatctagcatattttttttccacaatccataatatgatgacttgtgtacatggtgtgaataaaagtcagtccattgctgcatttggtattggttacgtgttactgtactttctgcatatattatctcttttatcatgtcgatgatttgattaatatttcttcaatttggatttattctttaattggttagtaatttcttctgtgaacttctagttagagcatgaactgctaaagaaatccaaaactttattttttacatggaaggaactttatcagagttttatttatttatttatttttatgttaaattgaactttaactgtttctatgttatgataactcttcttcagatatcagaagtcgattgacatttatgaagagatagctcgccaatccctcaacaataatttgctgaagtatggagttaaaggacaccttcttaatgctggcatctgccaactctgtaaagaggacgttgttgctataaccaatgcattagaacgatatcaggtctaagttttttcaatagttcacttctggagactggacagcttatttgttgctaaattattcagatatgtttttattttgcaggaactggatccaacattttcaggaacacgtgaatatagattgttggcggtaggtcactggttttgaaatttcgttatgaattttttatgaccaagtaaattggattagaatatttgaacttctttgtagctgtctcctgggtcataatgttttattatatttttgtatttatcatagcattgtgatagccctgttactactttgtttgctgatttactcatacatttgccagatgaaactgacatttttttttaatcctggtggataggacattgctgctgcaattgatgaagaagatgttgcaaagtttactgatgttgtcaaggaatttgatagtatgacccctctggtaagctccaaaagttgttaaataggataacttctagtggtgtttaacaaaaaaaaaaattccacttgtattttttatccacattttataacagaataatcataacctttcacaacttaattctcaattttcacagtaattaaatgtgtaattttaaaaaaatattttccttaacttaaacctgattgaaatttccccctgaaatttaagttctatttgattacctagagtgtaatttccgtgttttgtcacttaatcactgtgtaaagttaatttttttgcttacaaaggtgtcttgtttggaatgctaaaataacaagtacacgtgtcaccaaatttagtaggattaacatttgttgttttttgccataataaacggttgaacttaacatttgttgtacgtgtcatcaaattctacaaattgtgagctgcttagtgggttggacaaacattttagcaggtggtttcgattgcctgttgaatacgtgaaattaaaccaaggcaaaattataatttgtttcttttgtctgtgtttcactcatacacattgaatcttgatgatacacagccttgttaattgttatccttccaattttttttagtgtttttgagcatctattcttgttggtcatgtgttttcttcactcatgtacctggttcttttcctacaacgataaatatgtatcctttgttttttttttccaactaaatatgtaatttcaaatttctaatcaatcattgcttccaaaatactctctctgtttcaaaataagtattatcctatattgttttacaagaccaagaaaagctaatatatagatgaaagaaattagtaattttacaaaactaaccttagtattaatattatactgaaaaactaaattgacacttattaggggtgttagtgtaaaaaagcaattaatattacattgaaaagctaacatgatacttattttgggacaacttttttctttcaaatgcaacacttgttttggaacggagggaatactagatattgtgctcccttgtatgccctggacataacgtatttaactggtctggatgagtttatgaatgtcattaatttagggggagtcatttagaatagcttacctataagtactttctaacttttctcaattagtttcacagtgcaatttattaaaaatgtctgtatctaatcaacattgtctgtgtgcttgtgcaggattcttggaagaccacacttctcttaagggtgaaggaaaagctgaaagccaaagaacttgaggaggatgatcttacttgaattgtacctttaatattcctggtggttggacctattgtttgatgatttacattgtactactatgtgtgtctgtccagttgttcgtcttacacatccacttacagagtgtacctgctttggttttaattgaattggtctgactgaattcaaaaaatgagtttttaatgaggttgctggagtctgatcttatctacattattatgaattgaattactatctatacttgttttacaccaggtttatgcgaacctgttagcaatactaatccatgttactttatgcggataatccataaaaacagaaagaattaaccatcacaatttattgataagtatatgatagcatattttaccgagagttgaaatttgaaaataagtcgtttctgtatgatttttgcttattttgaccgacattaaatacctacctggtaaagaaggatggaacatatcaaggtagggtatttcttattacaagacaaacaaaaaatatagtaacaaactgggtgttaaaaaagtcgtgtaatgaatggacggtccgcaaccgcaaattatacctttgaactagaaaagtctatagcttcctttctttttcttttttccgttcctagactgttctactttttgtaaaggaaaagattcaaaagagagaacgcaaaataccacgcggcaattttttacttttttgcttgattatcttatcgtggaattccttttccaatctcaataactttttattttcaaatgtgtttttagattttatacttttgtcaatcaggttcacctactttattatattgataaacttggtcctcaaatttttaataacctgaaaaattattttcaattcattaagaaatcatgatttttcaaaattagaagtgactgaattcacatattttttaaagtttgagaactaaatttaacaatttaaaaatagagattcatcatgtttcacaaaaaatataaggactagaaatattttttcttcttcaacaatttactcttaacattaggctaaaatagaatatttgttcttacggtttgccactttaggaacaaaatttaacttaaaatacaaataaaggattaaaaatccattttaacttatttttaataaaatactgtatgatcattaatctaattaatatgtttttttcttgatgaaagtatgactttgttaatcataataatctaattatacgaagaatcgcgtgaccttatactcgtgcttggaaataaaagagagacatttgataaattgctttaacttttgatcttctttcttacgtagtagttttttgtcccacaaaatgaattttgcatgtattcagtgcttccttcttcggcttcactttttctggccggtggcagccggtaaccagtagtcatatttggatgttaaagagacagaaaatcttaatcaccgctcattgtttgactgcattgttacctgcgactgcgagtacgtggattcattcttgtttcgccaagtgtatgagtgcgtgtcagtgtgactcttttttgtaactttttcctttgtattagcgcttagacttttgattccaaaccatttttcttttctttgtttctgaaattttatcaatcaaacataactctgaggaaatcacacttccccggccgtcatgagtcagctaattaattggtatgtctaattttcaccaccaccttatcgggtcttcaaaatttaatgctattattctcagatttcttttcttgttcctacattctgactttgcatctgtcactgttctgagaactgaattttgttgaattattagaaaaatagaaatagattctgggttttcatttctagttttaaaattgtttattaagcatatgaacaccgtcaccactcaccatagctcaattctctgtctttatttttttatttatttgctttgatactttccccggtgcttatatggatgcatagaaatagaaaatttgctacagacttgtaaccttggcatagtttcttcatgtcttcttcgcagtatttttctgtacctatatcattgatgatacggttctgatttgatcgagaaagctcagttttttatcagaatggtttcggttgatgatgggattgtgaatcccaatgatgaaattgagaaatctaacgggagtaaagtgaatgagtttgcatctatggatatttcagcaactcaaaaatcatatctgaacagtgaagatcctcagagaaggcttcagggaaccttaataagttcttctgttactaataggataaactttcttaaatttggttctgcatctgccaaattcaaaaggcttgctactgagagagaccaggtttctatatctgtgccttctcctcgttcaaagagcctaagatcacgtttcagtggcatgtttgctcagaaacttgactgggcttcagtcaagaaaatgtgcatggaatggattagaaatccagtgaacatggccctttttgtgtggatcatttgtgtcgcggtttcgggtgctattctgttccttgtcatgacaggcatgttgaatggtgtgctaccaagaaagtctaagagaaatgcatggtttgaagtaaacaaccaaatactcaatgcagtgtttacactcatgtgtttgtaccaacaccctaagagattctaccaccttgttcttctgaccagatgaagaccaaatgacatctctagccttaggaaggtatattgcaagaatgtcacttacaagccccatgagtggacacatatgatggtagttgtcattctccttcatgttaactgttttgctcaatatgcactttgtggtctaaacttagggtataaaaggtccgagagacctgccattggagttggaatatgcatatcttttgcaattgctggtttgtacaccattcttagcccacttgggaaggactatgattgtgagatggatgaagaagcacaggttcaaattacagcttctcaagggaaagagcagctgagagagaaaccaactgagaagaaatattcatttgcatccaaagatcaacaaagggttgttgaaaatagaccaaagtggagtggaggaatacttgacatttggaacgatatttccttagcatatctctcacttttctgcaccttttgtgtgcttgggtggaatatgaagaggcttggctttggaaacatgtatgttcacattgccatttttatgctgttctgtatggctcctttctggatttttcttttggcttccgttaacatagatgatgacaatgttaggcaggctctagcagctgttggaatcattctttgttttcttggtttattgtatggtggattttggaggatccaaatgagaaagaggttcaatttaccagcctatgacttctgttttggcaaaccttcagcttctgattgcacactttggctaccctgttgctggtgctctctcgctcaagaagcgcgtaccaggaataactatgatcttgtagaagataaattctcaaggaaagaaactgatactagtgatcaaccatcaatttcacctttggctcgtgaagatgtagtgtcaaccagatctggcacaagttctcctatgggtagcactagcaactcttccccttatatgatgaaaacatctagttctccaaattcaagcaatgtcttaaagggatattacagtccagataagatgctatcaactttgaatgaagacaattgtgaaagaggtcaagatggaacaatgaaccccttatatgcacaaaaataatatcaaaatactatagacattaactctgtcttatcatcttttatgaatctcaatatatttctgtgcatatatcagcatcagcgtcactgaattccttggacattgacactgaacactcatgtatgagctggagatatttattgtctttattgaacaaattcaagaaaaagaagaagaaataagcctcgaactttgattcttaaaaatgtgtatttcattttaatatctaattctctaaaacttttactttaatttctaatttgatatgttgtcatataataaaatataatttagtttttctcatttcatttttattggtataaaaaattaaaaagaataatattttataataccttacacatcaacaaacaaagtgaagatttttatgcaataaaaaaattaagccattaatacttatactaaaatgaaggtttactcaaacaaattataaaaaaaaaataaataagtaagacattaatataatgtagatacccaacaacataaatggtcgacgtgtcacggcacacaatccaattttctttgctaaaatactataaagtataaacaaaagagtatatgattagcattaccaatgaacgttaaaaaaaaaaaaaaagcattaccaatgaagttggggccatacttcccttagtaccaaaaagaaaagcatatgaagttgggtttaacagaaaagagttagttctactgtgaaatttgtctaaatttaatatccggtcatatttaaaatagaattacctttaaaaaaaatacatgtgagaaactaaagaaaaattgtttaacattaaaaccatcgacactctataaatgatgccctatccacagaccactctttagtgtttttaataccctgactcagcaagcaatataatccacttactccccaaacctaaaaaatatacaaaagtcaaacaaaatgctatttatgtgaccattttaaatacaaggaaattggagtttcagatctttttttctttgcaaacttgccacctttgaagtgaaacataagacgaaatagatagtgacacactgacagtgacacctaaatagtagctacattgatgcattgtgtctagtgtaattccatgactcattgaggagcttttccatagatgaatagcatgtttatggtatgggactgtagagtagtggagagttgcttctgggggagtgcttatttggagcattggcaaatggcaattgccatccaaaacaatacaatacattacacatactgataaaatagtacagtggatatgatagaccatgcttatgtcttatgtgattcggattgattgcattccatattagaacagttgctattgttactatgtcatttgaatttaaatttgagaaagagttagtagtgaaattacatgtcatttaagcacaatcattatatattaaatttattaatttttataataattatatttaaaatcatataagtaatgattcataattatatgacaatctaaaatcaatacataatcatcaaattatttaaattttactgtcaatatgagaattttgccaataattaatatataaaatctcagggattttaatttattgagtttgtaatttttaaatttgaacctgaccgatgattaaaattaactcatatttttctcttccatttagtttggattgatccagtcatctggtagatctagatatgggttcactcttatgtgtattaactcgttatcattcattttttctttttgagaaaatgatatgctgaataattatacgcgaaacctcctttttcttatatggtaccatttgaaatatgagttagtcataaaagaaatttgaattataagttgataaaataagcatgctttcttttttcttaaatttttaatcattattattatgatgatggtttttgtttggaatcttagtcggtgccgtcagttgaatccgaaaagaatgaatagacagaagtgctttccgacccagagaaccaaacagtagctaactttgcgcttcttgttggtgttgttcgttgagatgcatagatggtgtgaaaattcatttttgctttttttacgaatgaatggaaacagattatctttttttaatttaaatttctttttgccttgtttcctgcaatgcatctttttttttttttttacgaagaaatggaaacagattaactttttttttataatttaaatcgttttcccttgtttcctgcaatacatctaattgcgtacaagatacaactacatttgtaattaacttttttttttattatttatatgtcactttaaaaatatagagtattatgaacggcgtctttacattttttcaattaaatgaccttggaaaattatgtacattatcaacgtataacctattttctcattattgttttatacacttgccataaaatttgataataaattgtttcatattaagcaaaataggctataattgaagtaattttctaactcatttttaatattaagcaaaatttaagtgaaatttattagatcactaaatcctattatttattacatattggtttacgtgagttatcgaaaaaaaaaaggttacgtaattttgcaatattcttttcccacattaattagcactaagacaaaaaaaaaaaaaaacattgtttttgggagtgaaaactgaaaagtctaaattgccaaaacttgtaatacctactatggttctacctagcttaccttgtggattgtagttaagctaaacccgttaaagacttaatgcaactaagtaaccaaaaaacaaagacaagcgaacgcatttgtatatacatgctttcacttatcactttttttttataaaaaaagaaaagatagcaacaaggtttgaacatatgatcatgtataaaaaatatgttttttatttattattttaccttaaatatgaaggaaataaaaatatacttttattgaagaatatttattaatgatataactaaaaatatgtcaatcatagtattgtaatgaataataatttaattgactaaaaaattaatgatataacaaattgtatccagtaaaagaaactaaaaatgtagtatcaatcattaataaatgataaaatcaaaatttacaaaacaacatattttagaattaccaaggtatcaaaatgttactatttcctcctccgtttcaaattatatgatattttaaaaagaaaaaaattgttcaaaaatagatattattttacaaaattaatgtaatattaaatatatatttttaaattattcttaatcaatattcagtgaaaataatatatagaaagaataaattaattgttaattaaagagataaatattatattaaaaattacttaatatttatttgaaattaatcgtatttattattattaagtgtgctttcaattctttaacgtggacaaatacttatttctgcataataagaatattaaaggtgaagagaatatccgatccacatatttttggtcaaactccttcagacatcagtgaagtccttaaaaactcaaattaagtcaaaaaagtaggcttgactactatcatcaatttgaacactcatgacgttgcaacatttaaaacccgcctactatttccatcttactccacttctattccatcgcccaatcaaaacccaacacgtcatcaaatcaaaaaatattcaaactagtaccgcccgcacccgatcgcaagcttcccggtacggaattcctatataaacccctcttccttcccattttaagacacaactccaacaaggcattgtttggtttggtttggttacttgaaaatctcgaatcgcttaattttgatttagttttccaccgcaacgcggaacctctttctcgaactggctaactctcaggcaagtggctcggacgctgattccagcaacacgcggctggtggttgcactgtatgacgccctaaactccggcgactccaacgccgtcgtcaagatcgtcgccgccgatctcgagtggtggttccatggtccgccctctcaccagtttttgatgcgcatgctcaccggcgactccgccgccgacaactccttccgattcgttccgcagtccatcgccgccttcggctccaccgtcatcgtcgagggctgcgactccgcccgcaacattgcctgggtccacgcctggaccgtcactgatgggatgatcactcaaatcagagagtacttcaacaccgccctcaccgtcactcgcatccacgattccggcgagattgttccggccagatccggcgccggccgtttgccctgcgtctgggagagcagcgtctccggtcgggtcgggaaatccgtccccggtttggttctcgcaatataaaatataaaataagtaattagggaaggacgaggtcacgtgttgccgttgctataataattaaataagggacttgtgcacgtggcggtgactggatcgatcggtttcagggaacattgatactttgtgttagtattggaggttagggagatgtgagagctttgttgttattggtgtggtttgttttgtttgcttgtgtgtttttcaccactatgggcgtattcaggtggttgtatctttcttttgttatttggagtgttgatgatgatgcaataagaatatctatggactatgcttttaagagttgggttgtgatgatgccaaatattctatttcgtctttgtcttctcattgttccaagttaattaattgggtaatgtgatttttaaatctaactgctcttggacacccagatgatccaagtcatctccttctcttctatatactaaaaaaacatttgctttctctaaaatgaggatttgtattttagagaacaaaaaaactaaatttgatgacaatttcaattattaatttcgtaattgatagttattattatattttatcctctaaaatgtcatttcctcattttacatgaaccaaatccagaaaaataaggattttttacttgcattaaatccaaatatggatataagattattacataactttttggtactaattcctcgcggatcatgtgtcattttagttagcataattccgacatttggatataaggatttattttattttattttctatcttcaataatttgtataaagtttgagagagaccattttgcacatatgtctttctctttttctctttttctttaatttaagggaaaataatcgatccaaacaattaaattaaataataagaattatataattttggtaattacaataattctaagtcacgaacagaaaatgttagactcatttttttaactttttggaagtggtggggctaagatccttcaggaaaattccaaaagggatgcaactgaaagagggattagcaaaattcctcttcgataatttaagaaagtgaaagataaatttggttctactatatgatgtgatgttgcgctttacatatgctcgttgcttggtgcatacttgattgaaaagactcaattttagggcataaacaatacaatacccttttacattacatcaaaacttctaataagttgtttcaattcgtgcgtgtattgtctatttatcaaattgccaacaaccctaaattatgatttaattggtctaagagattatgtcaatggtgtaatcggaattgaggtagagatgcgcctggtatattgtctaaccaataaaccaattgaatttggcaacttgaatcaaatttcaaatatcatctttgtaagctcagctactaaaaataagtagaatgcatctgtttttgttttgtcctctaatattggtctgaaatatctattaattttgttattattaattaatttttgttaaaaaatttaattgattatttttgttgaaatatttcttattaattatatttttttatttacagaacttaaatctcttgtttaaaaagaagattaagatccaacaccttgtttaaagagattaaaaaatttgatatcactaccaattgactttttggtaaatatgtaggatgtataataatgataattagagtttttatgaaaaatcttttaggggcaaaaaattatttttaagaaatatatatacgacttttctagaatacgtggaggcacagctaacaggaagctggagtaaggtccaccatgtcttgggctaatacaacataaacctcttcacttccttttaaattgcaataatcacatgcatcgcatcgtaacgcatggtcttgttttttgttagatgattggtcactttcccacggtcgcggtagaatcagccaccaccatttcttttttcttctaggacccatttgtcagaccaggattcgtggactcaagatattcactgtactatgtgcattcattttgctacatgtttaggaacaaaagagaagagaatctctatgttaagtgctaattacacataaccagccagataggggcatccattgatatctttgtttttccctctcatattgtcacgtttttatatattcttttacatcttaggaaggaactataaattaaaaacacccatgtgcgtgtcccttttaaacttaataatttaggtggatgcatgatctggaactcaattaagtatagcttaatttatagttttattttggagcgtgctaaataaaataattaaactccatgcagagcaggattttattccttcgggataattgtgtttactgattagtgtgcatgaacaaaagctgcggctctttgttttatacatttgtttgatactttgactagataaaagattaaaaaaaagttacagcagaaaataataaatgtatctgtgaatggaattataattatattgtttcaaaaaagaagcaaagggtcaaattttcctatacaacacaacaatttaacatctatctccttgcatcagacaccaaaccacaaatccggcactggttattcattgatcaattcgaactcaaacaagaagacacaaataattcaccgtctcttatggatgacttcgcaaatccaagacgtaacttatttattggaatttgagttcagacagaaagacacaaacaaatggattacaagcctcattattccgtcaggaaaaaaaataggtggttttgtttttctcttttcactatgtctagtagagtccacaccacatactcactagtacaaagataacaagataaacagttgaacacccgtactatttcaacgaaaaaaataataaacgatccaaatttaacaactaatattgtggagttgttaaatcatagctataggtcaatttgcacaaggaatgagagatccattagaaccaattagtgttttccactagtttatgacatctagttctcatagaactttaaactagttgtaactaatttcacaaatctaaagataaagttattaaagcttaaattttagacttattaataaaaaaaataccacatatattgataaaaaaaaaagcccaacatatacatctttcattttaagtagaggagtgcttcccccaaaaaccctagaaacaataacaccctaggaatcctagtaacagaacacgacaacacgtaccctttaattttaaggggacttctccctcctccttggagagcttctacctccattggaagacttctctcccatctcaggaggttttcttttccaacatcacgctccccctcaatccaccacctcttttcctcatctttcttttttcctttttcagttgctattctcatctcttctctagctttataatttttttgtttgtttttttaacattcccattattttttattcctatcacatttctcctttacgatggagcttgttagaggcctatatattgcagatggatctaacagaatgaaagatcgatagaaaatattagaaaaaatgtcattaacattgaaaaaaaaacatttcttaaaaattatttttaagtctcacttttgctagctaacctcgagatcacaaattatatataactttttttttatcgtgctctgttgcaatttcatctcaaatttattttgataattaatttaatttttaattatgatttttatttgtctatgaatattgatatatcaatacgactttaaacattaaactaattgctcaaatagtttacacaagtactaatgaggtcaaggttgaacaactaaccttgatcgaattctagattgctctaatggttcgtttagaagggatgaaaatgcattttctatggattaagatttgggatgtttagatgacggtgctgctttcaacacacctgaaacattgtgaatatatttttaaaaaaatctcattatatagttaataaaaaatattaacgtcatcatttaaataaacatttaataaaagaatatgaagaatttgacataaatattttcacttggtgcatgtttggtaacatgtgagttgaactcgatacgattttttaaaatggtttttgtatttatttatttttaaaatatattttttaccaccaattcaaaaacactatactatccaacaacacgtgcattaactaacatgggatttgttaagtttgatatgtgatcttgagtttttgagacctcactatttagttatattaaatatttgaaagaggaaaaataatttgcaatccataataatcttacaaaagtgaagtaaaattatttttttataaaagatacatgtgacaatgttccaaaacacactattataattattattatctaactcatatgcattgacaatttgattcagtggagaggagagagaagttatcacgttaagtggggattagttaattaagtgcacaaatacgtcaccttcgttttcaatatgccattctgcttttcctcccacgttttttcaagccgttcgatttgttttctgtaattgttttcaaccaaggaagagaataaatccaataaaaggacatactgtcggggtagtgatcgtttgatgatgatattgataacattggcatcttggagaatatcgcataaacacaattttgattttctctttataggagtttccctgaactttgatcattatacgtattcacataacagaatccattttttttttaaaaaaaaaaggatccatatttcatttcctcttaattatttgcttccttttcccatgtaggtgactaggtggtgttttggccagggtcccagacttgctaaattgcacagttaaggaatattttcatcattggattccactaacaaaccctgaagagtcttatcaatatgaattatttactatgccaccatatatgatatatgttaaacactaattagtgatctgatgctaattgtgaagtgctgagaaattttaagctacgaaagcgatcgtatgaaagataagtggttttcagcataaaaattaaaacatattataaaaaaataataacacatgaatcattccttaatttaaatattttatcgacaattcttatttttttatttttttctcacatcataaatttcattatatttatattttttttctctctttctaaacgtaggaattaagataatatatgctatgtatatcaaacactttcgattataaagaaaaatatttgagatatttagaaaagtttgtacaatgatttagaatgggagaactacttcaccgaattctgtggtaaagaagggtgacctcagttttttctttgcttatttcttcagttaattattactactgttattattgcatgtacacccaataagtacttaaattaaagaggcaaaaaataaagaaaatctaattttattaatgtaatatttttatttttaatttttagaaggttacaggacacatcagttaaaagagtggatgtcatgatttttagaacaaaaaaagagaaaagaggaaaaccttaaataacattgaaaacactcattaaaaaagacttgagactttgaaaataattcttaaaccttaatttttaactgtgttaaatgatgtcatgtgatttatataattgatttcacttaataataagacttttgctgttattgttgtttatttattttgtttattttaacttgcacagttggtgcgtagaataaaaaagaaattaatcgttataactatagctatcaatacaagtagatcaagctacaagaagtttttatcatagaattgaattagttactagttgggtgtgtttggttcacgcattaataacatagttttcatatctggatatatggaagtgatctcttatagctttttgcatcttttattcaatgaatatgatcaatcactgcacaatgcatttccgaacacttggttagtggttggaggaatctagtctccgaaattgtccatgactttaatttaaattaggtgttacgttgttatcatttatcaagcacccgttcccgtcacttctggttaaaatccattagcctttgctgctaaaaaaacttagaatttatcttagtggggaacattttgatacaacctaaagtaagcattcaagttttgaagacagtaagcaacttaaattttatggctctctttactaatgacgccattagttaaccacacgactcaaaatttaagttatttgatatttacgtttaataacataacactacctcatcccaatagccaaatatgtatatatatatatatatataaaattgagagaaattttactattttcacgtcttggtcagttccattcttgtagaaagtcatttcctttgttttttctgcggcttccacatcactgtcgacatttttccacgacctttacttttttttctctagcttatgagataagataagaggcagcctattcatatcacattatcatataccaccactgatatatgaatttttaagcctgtgttgcgtccttatcataaatttacatataaccctacgtgtgttatctatattagaaactgaaatatgttattaacattaatatacaccactgcataggataagtactactttcgactttcaaagattaagaaaaatgaggtgtccatatcaaaacagtgggataaaattatatattaagactaattcaaaatgaatttaaatcgggcttagttttcacatgcttaaatatttccatttctatatcttagacttccaattccaatgttgaattgtggaagtaaattagcatatataggaactattttaagggatgaaggcgagcatactactcctaataataaaggtatctgaatgaactcaaatgaagaataagagataacttgtaaaaaaaaactattagaattgagagaatattattttatcaataaatataaagtattttttattatttatatattttctataactaccataacagaaaactaattacttctaactcattataacaaacttagtttagttaggtatcactaactcaaattacactcggatgggtaatacctcaagacatcaattggcgtaatgtcatagtcatagtcatataattctcagatcttgagaacaatacaagcaagattctgaaatgacatcggatcggtatcttattccatggctagcctttttaattggttaaactgaagaagaaaaaaatagcacaagaaataaagagagagatggaatcagatcgcgtatatgctcattgctgtaagagaataaaattcataaacgtgctagtttttaagaatattcgtagatcagttggaatgtgacaatcgtggttgctgaaagttttggaataatggtctaaaatggccaattttatggcagagctaagatgctttagtctaccggggtgtcaagacaatctagtacttcagttggttgattaagcctgtgtaaattattataaaatttgtaatattatctttaattcttatgaaaaaaaaataagaatatattgggagtggattaacacatcattcagcttatttttttaaatgaaattagataaagatacattttttaagaaaattaggtaatttaaataatatcatctataaaagtacttgcctttttttatgtattcatgtatcttacttatttgatgaatgatgataaatgttaaattaatattttctctttgttaattcaagaaatattaaaacattgagatatataaaaatcattactattaaaatattatttttattaattaaatatctttatatttaaaattttaaacgtatgcaattcttatgttttatcatcaaaatcttttctaaagttaaatcaatcttttctgcgtatttttatttatatttaagataccttatatttaaaagtacgtattactcatgcataaaatactttctactttttttaaataaaatactttttattttttataatttttttatatctataataatagtctaaagtattcattaattttattgataactaattcttactgtagaatctgatcaatcatctttagtgtctttcaaattacatttaatttattcgtaagactaaaacatgagattttgtttaattagatcaaactcaataccacttgaataaattacttgttagtattacttttcatattatgttcgcaagctaaaaattatagcattagttgaatttcatctagccatttacaaactttattcaatgggccaatttctatgaaaaaaaatattttatcctctaaatgttgtatatattttggaatttgagagaaacaaaaaaaaagagaaagattgtgaatgtgatagatgatataataaaaatataaaaaaaaaatagaaaatgatataaaatagatgtaaattttagggtgcccaaaataattgaatctatgtgtagtaataataatggaaaaataatataaaaatattataaaaagtgcaacaatttcttaactatagtctataggttacttaaagtagggttgttaaaatgagtagatccgtttaactgagtcagctaattaaaatgtgttgattgaatttgaaaattttgaactcaatttaattttgattttactttattcactccaaagatttgtttgaacgtaaagttgtaatgagactagttcgttagtccattttcttcttaagcaaatatatatcacccattcattaaattgagctaggttttgaattaaattttacaaaatttgaaatagtcaaatttgtcaatccaacttgattagaaattctcatttaatgaatgaggggaactagcctgaattgctacttgctatatacctgaagtcttactttcattgtcatattataattatggagtgagaaacaaattattttaaaacaatcattaatttaatgttttaatgtaatattaattattttttatttatatctcttataatattaataataaacatcaaaatttataaataaattaataataatataagattaattttataaaattattattttttaatttgtataaaataacttaagattagtattattttaaaagggatggagtatgatatgcaatataaagcaataaaatcatatatatctgccatgtcagcatgtataatgacatctaaattaaaatggctggtggataagattttttgaacttcgcttcttatctctcaacaactggaggctattatgtccactttctacgacatcaaacacatgttaggtgcatttggttgcaatttgcaatctataggattaggagggtgtttggtatgtagcttacaagactatttgctttgaattttcaagtgaccgtatccagagtttttgctaatatctcatcagatattagacatttagttttcattagtatctatctccgcgcaatgcaagagacttgacgttaagaatttatgagaaccacaggtggaactgcattagcatccttcaattttcacgaaaatgatatctattactcaaactaaagtggcattttaagctggaattttaagaatcataaattttttgagctttgtttgtgtggagtaaagactcaaatgagaatacttattttatctcacttatttaagtagaaagaggtcaattaaggaaaaaaaaaactcatttgaaaggaaaaaaataattacaaattattgagagagaaatgagagagaaaatcattgtgattttcgtacactcaccgatttttagattacaactgcggattctttggattaggttgattgttagacagcaggttctacatatataatacttcaaattgtttgatgagatcgttaaaaagatatttgaagagagagataaatgtttttcattttctgttttatattttgggatttcatcttcttgtctctattgtatcaattgggggtctgttttgatttggctgtttgtagcacgtttcgatgcacttgttgaagactttcttgtaactttattgattatagtgaaattatttctttggtataaatgatccgtgatttttacccttgcattaagggatttttcactttaaacaaattgtgtctcttgtgcgcttttaatttctattttgctctctttatattttagcctgctccccaagtttggaccaatttatttctgctgcctatattactttgttattgtgttggtatattttcttcatcaaaaaatatccatttgtgctttaaattttgggtagttttgtttcttgctccacaaatttttgcagttttagtggaaaggcccaaccaatattctcaacattttgggccttcctcgaacaaggacccgtaagaatagaagtttctaaaatggacttgtaattggtg

SEQ ID NO: 69 - DNA, 23 bp, Glycine max
ggcaaggcacactgcggatgagg

SEQ ID NO: 70 - DNA, 23 bp, Glycine max
gtacgctggcgtcatgagggagg

SEQ ID NO: 71 - DNA, 23 bp, Glycine max
ggcggccggagacatgccggagg

SEQ ID NO: 72 - DNA, 23 bp, Glycine max
ggaaattgctgaattgtacgagg

SEQ ID NO: 73 - DNA, 23 bp, Glycine max
gatcttaggctctttgaacgagg

SEQ ID NO: 74 - DNA, 23 bp, Glycine max
gggaagcttgcgatcgggtgcgg

SEQ ID NO: 75 - DNA, 23 bp, Glycine max
gaatcggaaggagttgtcggcgg

SEQ ID NO: 76 - DNA, 23 bp, Glycine max
ggctgattctaccgcgaccgtgg

SEQ ID NO: 77 - protein, 1387 aa, Artificial sequence
  Synthetic
  MISC_FEATURE (1)..(10): nuclear localization sequence
  MISC_FEATURE (1378)..(1387): nuclear localization sequence
GSKKRRIKQDMDKKYSIGLDIGTNSVGWAVITDDYKVPSKKFKVLGNTDRHSIKKNLIGALLFGSGETAEATRLKRTARRRYTRRKNRICYLQEIFSNEMAKVDDSFFHRLEESFLVEEDKKHERHPIFGNIVDEVAYHEKYPTIYHLRKKLADSTDKADLRLIYLALAHMIKFRGHFLIEGDLNPDNSDVDKLFIQLVQIYNQLFEENPINASRVDAKAILSARLSKSRRLENLIAQLPGEKRNGLFGNLIALSLGLTPNFKSNFDLAEDAKLQLSKDTYDDDLDNLLAQIGDQYADLFLAAKNLSDAILLSDILRVNSEITKAPLSASMIKRYDEHHQDLTLLKALVRQQLPEKYKEIFFDQSKNGYAGYIDGGASQEEFYKFIKPILEKMDGTEELLVKLNREDLLRKQRTFDNGSIPHQIHLGELHAILRRQEDFYPFLKDNREKIEKILTFRIPYYVGPLARGNSRFAWMTRKSEETITPWNFEEVVDKGASAQSFIERMTNFDKNLPNEKVLPKHSLLYEYFTVYNELTKVKYVTEGMRKPAFLSGEQKKAIVDLLFKTNRKVTVKQLKEDYFKKIECFDSVEISGVEDRFNASLGAYHDLLKIIKDKDFLDNEENEDILEDIVLTLTLFEDRGMIEERLKTYAHLFDDKVMKQLKRRRYTGWGRLSRKLINGIRDKQSGKTILDFLKSDGFANRNFMQLIHDDSLTFKEDIQKAQVSGQGHSLHEQIANLAGSPAIKKGILQTVKIVDELVKVMGHKPENIVIEMARENQTTQKGQKNSRERMKRIEEGIKELGSQILKEHPVENTQLQNEKLYLYYLQNGRDMYVDQELDINRLSDYDVDHIVPQSFIKDDSIDNKVLTRSDKNRGKSDNVPSEEVVKKMKNYWRQLLNAKLITQRKFDNLTKAERGGLSELDKAGFIKRQLVETRQITKHVAQILDSRMNTKYDENDKLIREVKVITLKSKLVSDFRKDFQFYKVREINNYHHAHDAYLNAVVGTALIKKYPKLESEFVYGDYKVYDVRKMIAKSEQEIGKATAKYFFYSNIMNFFKTEITLANGEIRKRPLIETNGETGEIVWDKGRDFATVRKVLSMPQVNIVKKTEVQTGGFSKESILPKRNSDKLIARKKDWDPKKYGGFDSPTVAYSVLVVAKVEKGKSKKLKSVKELLGITIMERSSFEKNPIDFLEAKGYKEVKKDLIIKLPKYSLFELENGRKRMLASAGELQKGNELALPSKYVNFLYLASHYEKLKGSPEDNEQKQLFVEQHKHYLDEIIEQISEFSKRVILADANLDKVLSAYNKHRDKPIREQAENIIHLFTLTNLGAPAAFKYFDTTIDRKRYTSTKEVLDATLIHQSITGLYETRIDLSQLGGDGSKKRRIKQD

SEQ ID NO: 78 - DNA, 23 bp, Artificial sequence
  Synthetic
  misc_feature (2)..(19): n is a, c, g, or t
  misc_feature (21)..(21): n is a, c, g, or t
gnnnnnnnnnnnnnnnnnngngg

SEQ ID NO: 79 - DNA, 23 bp, Artificial sequence
  Synthetic
  misc_feature (1)..(21): n is a, c, g, or t
nnnnnnnnnnnnnnnnnnnnngg

SEQ ID NO: 80 - DNA, 300 bp, Artificial sequence
  Synthetic
aagctaaaagttgcaaaagaaatggcagggctataaggctcacctactcctggatttaccaaattttggttcgtccctatactcgaaaaataaaacaaaataaatttcagtatcttcgtttttgtatgctttgactgtgaggcgaggccaactttcttcttctgtctgagatgaattttgtttgcctcctgtgaaggatgtatcattcaaagtgaatgttttgcaactgccagtagtcccacatcgaccaaatattcttattacagtgtgtttatatagcacctggagaaggaatgggtt

SEQ ID NO: 81 - DNA, 300 bp, Artificial sequence
  Synthetic
aaatggtaaaatgtcaaatcaaaactaggctgcagtatgcagagcagagtcatgatgatactacttactacaccgattcttgtgtgcagaaaaatatgttaaaataattgaatctttctctagccaaatttgacaacaatgtacaccgttcatattgagagacgatgcttcttgtttgctttcggtggaagctgcatatactcaacattactccttcagcgagttttccaactgagtcccacattgcccagacctaacacggtattcttgtttataatgaaatgtgccaccacatggatt

SEQ ID NO: 82 - DNA, 84 bp, Artificial sequence
  Synthetic
gttttagagctagaaatagcaagttaaaataaggctagtccgttatcaacttgaaaaagtggcaccgagtcggtgctttttttt